European Patent Specification EP 3 653 212 B1, published April 26, 2023. Title: CHIMERIC ANTIGEN RECEPTOR-EXPRESISNG T CELLS AS ANTI-CANCER THERAPEUTICS. Applicant: LOW, Philip CHU, Haiyan LEE, Yong G. The sequence listing filed with the application follows.

SEQUENCE LISTING (2 sequences)

SEQ ID NO: 1 - DNA, 8561 bp, Artificial Sequence
  lentivirus expression construct encoding a chimeric antigen receptor
acgcgtgtagtcttatgcaatactcttgtagtcttgcaacatggtaacgatgagttagcaacatgccttacaaggagagaaaaagcaccgtgcatgccgattggtggaagtaaggtggtacgatcgtgccttattaggaaggcaacagacgggtctgacatggattggacgaaccactgaattgccgcattgcagagatattgtatttaagtgcctagctcgatacataaacgggtctctctggttagaccagatctgagcctgggagctctctggctaactagggaacccactgcttaagcctcaataaagcttgccttgagtgcttcaagtagtgtgtgcccgtctgttgtgtgactctggtaactagagatccctcagacccttttagtcagtgtggaaaatctctagcagtggcgcccgaacagggacttgaaagcgaaagggaaaccagaggagctctctcgacgcaggactcggcttgctgaagcgcgcacggcaagaggcgaggggcggcgactggtgagtacgccaaaaattttgactagcggaggctagaaggagagagatgggtgcgagagcgtcagtattaagcgggggagaattagatcgcgatgggaaaaaattcggttaaggccagggggaaagaaaaaatataaattaaaacatatagtatgggcaagcagggagctagaacgattcgcagttaatcctggcctgttagaaacatcagaaggctgtagacaaatactgggacagctacaaccatcccttcagacaggatcagaagaacttagatcattatataatacagtagcaaccctctattgtgtgcatcaaaggatagagataaaagacaccaaggaagctttagacaagatagaggaagagcaaaacaaaagtaagaccaccgcacagcaagcggccactgatcttcagacctggaggaggagatatgagggacaattggagaagtgaattatataaatataaagtagtaaaaattgaaccattaggagtagcacccaccaaggcaaagagaagagtggtgcagagagaaaaaagagcagtgggaataggagctttgttccttgggttcttgggagcagcaggaagcactatgggcgcagcgtcaatgacgctgacggtacaggccagacaattattgtctggtatagtgcagcagcagaacaatttgctgagggctattgaggcgcaacagcatctgttgcaactcacagtctggggcatcaagcagctccaggcaagaatcctggctgtggaaagatacctaaaggatcaacagctcctggggatttggggttgctctggaaaactcatttgcaccactgctgtgccttggaatgctagttggagtaataaatctctggaacagatttggaatcacacgacctggatggagtgggacagagaaattaacaattacacaagcttaatacactccttaattgaagaatcgcaaaaccagcaagaaaagaatgaacaagaattattggaattagataaatgggcaagtttgtggaattggtttaacataacaaattggctgtggtatataaaattattcataatgatagtaggaggcttggtaggtttaagaatagtttttgctgtactttctatagtgaatagagttaggcagggatattcaccattatcgtttcagacccacctcccaaccccgaggggacccgacaggcccgaaggaatagaagaagaaggtggagagagagacagagacagatccattcgattagtgaacggatctcgacggtatcggttaacttttaaaagaaaaggggggattggggggtacagtgcaggggaaagaatagtagacataatagcaacagacatacaaactaaagaattacaaaaacaaattacaaaattcaaaattttatcgatactagtaaggatctgcgatcgctccggtgcccgtcagtgggcagagcgcacatcgcccacagtccccgagaagttggggggaggggtcggcaattgaacgggtgcctagagaaggtggcgcggggtaaactgggaaagtgatgtcgtgtactggctccgcctttttcccgagggtgggggagaaccgtatataagtgcagtagtcgccgtgaacgttctttttcgcaacgggtttgccgccagaacacagctgaagcttcgaggggctcgcatctctccttcacgcgcccgccgccctacctgaggccgccatccacgccggttgagtcgcgttctgccgcctcccgcctgtggtgcctcctgaactgcgtccgccgtctaggtaagtttaaagctcaggtcgagaccgggcctttgtccggcgctcccttggagcctacctagactcagccggctctccacgctttgcctgaccctgcttgctcaactctacgtctttgtttcgttttctgttctgcgccgttacagatccaagctgtgaccggcgcctactctagagctagcgaattcgaatttaaatcggatccgcggccgccgactgtgccttctagttgccagccatctgttgtttgcccctcccccgtgccttccttgaccctggaaggtgccactcccactgtcctttcctaataaaatgaggaaattgcatcgcattgtctgagtaggtgtcattctattctggggggtggggtggggcaggacagcaagggggaggattgggaagacaatagcaggcatgctggggatgcggtgggctctatggcctctggcctcgcacacattccacatccaccggtaggcgccaaccggctccgttctttggtggccccttcgcgccaccttctactcctcccctagtcaggaagttcccccccgccccgcagctcgcgtcgtgcaggacgtgacaaatggaagtagcacgtctcactagtctcgtgcagatggacagcaccgctgagcaatggaagcgggtaggcctttggggcagcggccaatagcagctttgctccttcgctttctgggctcagaggctgggaaggggtgggtccgggggcgggctcaggggcgggctcaggggcggggcgggcgcccgaaggtcctccggaggcccggcattctgcacgcttcaaaagcgcacgtctgccgcgctgttctcctcttcctcatctccgggcctttcgacctgcatctagagccgccatggcttacccatacgatgttccagattacgctagtttggtgaggcagcagagaccgatggagagcgacgagagcggcctgcccgccatggagatcgagtgccgcatcaccggcaccctgaacggcgtggagttcgagctggtgggcggcggagagggcacccccaagcagggccgcatgaccaacaagatgaagagcaccaaaggcgccctgaccttcagcccctacctgctgagccacgtgatgggctacggcttctaccacttcggcacctaccccagcggctacgagaaccccttcctgcacgccatcaacaacggcggctacaccaacacccgcatcgagaagtacgaggacggcggcgtgctgcacgtgagcttcagctaccgctacgaggccggccgcgtgatcggcgacttcaaggtggtgggcaccggcttccccgaggacagcgtgatcttcaccgacaagatcatccgcagcaacgccaccgtggagcacctgcaccccatgggcgataacgtgctggtgggcagcttcgcccgcaccttcagcctgcgcgacggcggctactacagcttcgtggtggacagccacatgcacttcaagagcgccatccaccccagcatcctgcagaacgggggccccatgttcgccttccgccgcgtggaggagctgcacagcaacaccgagctgggcatcgtggagtaccagcacgccttcaagacccccatcgccttcgccagatcccgcgctcagtcgtccaattctgccgtggacggcaccgccggacccggctccaccggatctcgcgagggcagaggaagtcttctaacatgcggtgacgtggaggagaatcccggccctatgaccgagtacaagcccacggtgcgcctcgccacccgcgacgacgtccccagggccgtacgcaccctcgccgccgcgttcgccgactaccccgccacgcgccacaccgtcgatccggaccgccacatcgagcgggtcaccgagctgcaagaactcttcctcacgcgcgtcgggctcgacatcggcaaggtgtgggtcgcggacgacggcgccgcggtggcggtctggaccacgccggagagcgtcgaagcgggggcggtgttcgccgagatcggcccgcgcatggccgagttgagcggttcccggctggccgcgcagcaacagatggaaggcctcctggcgccgcaccggcccaaggagcccgcgtggttcctggccaccgtcggcgtctcgcccgaccaccagggcaagggtctgggcagcgccgtcgtgctccccggagtggaggcggccgagcgcgccggggtgcccgccttcctggagacctccgcgccccgcaacctccccttctacgagcggctcggcttcaccgtcaccgccgacgtcgaggtgcccgaaggaccgcgcacctggtgcatgacccgcaagcccggtgcctgaaatcaacctctggattacaaaatttgtgaaagattgactggtattcttaactatgttgctccttttacgctatgtggatacgctgctttaatgcctttgtatcatgctattgcttcccgtatggctttcattttctcctccttgtataaatcctggttgctgtctctttatgaggagttgtggcccgttgtcaggcaacgtggcgtggtgtgcactgtgtttgctgacgcaacccccactggttggggcattgccaccacctgtcagctcctttccgggactttcgctttccccctccctattgccacggcggaactcatcgccgcctgccttgcccgctgctggacaggggctcggctgttgggcactgacaattccgtggtgttgtcggggaaatcatcgtcctttccttggctgctcgcctgtgttgccacctggattctgcgcgggacgtccttctgctacgtcccttcggccctcaatccagcggaccttccttcccgcggcctgctgccggctctgcggcctcttccgcgtctccgccttcgccctcagacgagtcggatctccctttggccgcctccccgcctggtacctttaagaccaatgacttacaaggcagctgtagatcttagccactttttaaaagaaaaggggggactggaagggctaattcactcccaacgaagataagatctgctttttgcttgtactgggtctctctggttagaccagatctgagcctgggagctctctggctaactagggaacccactgcttaagcctcaataaagcttgccttgagtgcttcaagtagtgtgtgcccgtctgttgtgtgactctggtaactagagatccctcagacccttttagtcagtgtggaaaatctctagcagtagtagttcatgtcatcttattattcagtatttataacttgcaaagaaatgaatatcagagagtgagaggaacttgtttattgcagcttataatggttacaaataaagcaatagcatcacaaatttcacaaataaagcatttttttcactgcattctagttgtggtttgtccaaactcatcaatgtatcttatcatgtctggctctagctatcccgcccctaactccgcccagttccgcccattctccgccccatggctgactaattttttttatttatgcagaggccgaggccgcctcggcctctgagctattccagaagtagtgaggaggcttttttggaggcctagacttttgcagagacggcccaaattcgtaatcatggtcatagctgtttcctgtgtgaaattgttatccgctcacaattccacacaacatacgagccggaagcataaagtgtaaagcctggggtgcctaatgagtgagctaactcacattaattgcgttgcgctcactgcccgctttccagtcgggaaacctgtcgtgccagctgcattaatgaatcggccaacgcgcggggagaggcggtttgcgtattgggcgctcttccgcttcctcgctcactgactcgctgcgctcggtcgttcggctgcggcgagcggtatcagctcactcaaaggcggtaatacggttatccacagaatcaggggataacgcaggaaagaacatgtgagcaaaaggccagcaaaaggccaggaaccgtaaaaaggccgcgttgctggcgtttttccataggctccgcccccctgacgagcatcacaaaaatcgacgctcaagtcagaggtggcgaaacccgacaggactataaagataccaggcgtttccccctggaagctccctcgtgcgctctcctgttccgaccctgccgcttaccggatacctgtccgcctttctcccttcgggaagcgtggcgctttctcatagctcacgctgtaggtatctcagttcggtgtaggtcgttcgctccaagctgggctgtgtgcacgaaccccccgttcagcccgaccgctgcgccttatccggtaactatcgtcttgagtccaacccggtaagacacgacttatcgccactggcagcagccactggtaacaggattagcagagcgaggtatgtaggcggtgctacagagttcttgaagtggtggcctaactacggctacactagaaggacagtatttggtatctgcgctctgctgaagccagttaccttcggaaaaagagttggtagctcttgatccggcaaacaaaccaccgctggtagcggtggtttttttgtttgcaagcagcagattacgcgcagaaaaaaaggatctcaagaagatcctttgatcttttctacggggtctgacgctcagtggaacgaaaactcacgttaagggattttggtcatgagattatcaaaaaggatcttcacctagatccttttaaattaaaaatgaagttttaaatcaatctaaagtatatatgagtaaacttggtctgacagttaccaatgcttaatcagtgaggcacctatctcagcgatctgtctatttcgttcatccatagttgcctgactccccgtcgtgtagataactacgatacgggagggcttaccatctggccccagtgctgcaatgataccgcgagacccacgctcaccggctccagatttatcagcaataaaccagccagccggaagggccgagcgcagaagtggtcctgcaactttatccgcctccatccagtctattaattgttgccgggaagctagagtaagtagttcgccagttaatagtttgcgcaacgttgttgccattgctacaggcatcgtggtgtcacgctcgtcgtttggtatggcttcattcagctccggttcccaacgatcaaggcgagttacatgatcccccatgttgtgcaaaaaagcggttagctccttcggtcctccgatcgttgtcagaagtaagttggccgcagtgttatcactcatggttatggcagcactgcataattctcttactgtcatgccatccgtaagatgcttttctgtgactggtgagtactcaaccaagtcattctgagaatagtgtatgcggcgaccgagttgctcttgcccggcgtcaatacgggataataccgcgccacatagcagaactttaaaagtgctcatcattggaaaacgttcttcggggcgaaaactctcaaggatcttaccgctgttgagatccagttcgatgtaacccactcgtgcacccaactgatcttcagcatcttttactttcaccagcgtttctgggtgagcaaaaacaggaaggcaaaatgccgcaaaaaagggaataagggcgacacggaaatgttgaatactcatactcttcctttttcaatattattgaagcatttatcagggttattgtctcatgagcggatacatatttgaatgtatttagaaaaataaacaaataggggttccgcgcacatttccccgaaaagtgccacctgacgtctaagaaaccattattatcatgacattaacctataaaaataggcgtatcacgaggccctttcgtctcgcgcgtttcggtgatgacggtgaaaacctctgacacatgcagctcccggagacggtcacagcttgtctgtaagcggatgccgggagcagacaagcccgtcagggcgcgtcagcgggtgttggcgggtgtcggggctggcttaactatgcggcatcagagcagattgtactgagagtgcaccatatgcggtgtgaaataccgcacagatgcgtaaggagaaaataccgcatcaggcgccattcgccattcaggctgcgcaactgttgggaagggcgatcggtgcgggcctcttcgctattacgccagctggcgaaagggggatgtgctgcaaggcgattaagttgggtaacgccagggttttcccagtcacgacgttgtaaaacgacggccagtgccaagctg

SEQ ID NO: 2 - DNA, 1533 bp, Artificial Sequence
  polynucleotide sequence encoding chimeric antigen receptor CAR4-1BBZ
atggcctcaccgttgacccgctttctgtcgctgaacctgctgctgctgggtgagtcgattatcctggggagtggagaagctgatgtcgtgatgacccagacccccctcagcctcccagtgtccctcggtgaccaggcttctattagttgcagatccagccagtccctcgtgcactctaacggtaatacctacctgagatggtatctccagaagcccggacagagccctaaggtgctgatctacaaagtctccaaccgggtgtctggagtccctgaccgcttctcagggagcggttccggcaccgacttcaccctgaagatcaaccgggtggaggccgaagacctcggcgtctatttctgctctcagagtacacatgtgccctggaccttcggcggagggaccaagctggagatcaaaagctccgcagacgatgccaagaaagatgccgctaagaaagacgatgctaagaaagacgatgcaaagaaagacggtggcgtgaagctggatgaaaccggaggaggtctcgtccagccaggaggagccatgaagctgagttgcgtgaccagcggattcacctttgggcactactggatgaactgggtgcgacagtccccagagaaggggctcgaatgggtcgctcagttcaggaacaaaccctacaattatgagacatactattcagacagcgtgaagggcaggtttactatcagtagagacgattccaaatctagcgtgtacctgcagatgaacaatctcagggtcgaagatacaggcatctactattgcacaggggcatcctatggtatggagtatctcggtcaggggacaagcgtcacagtcagtgtgaactctactactaccaagccagtgctgcgaactccctcacctgtgcaccctaccgggacatctcagccccagagaccagaagattgtcggccccgtggctcagtgaaggggaccggattggacttcgcctgtgatatttacatctgggcacccttggccggaatctgcgtggcccttctgctgtccttgatcatcactctcatctctgtgctcaaatggatcaggaaaaaattcccccacatattcaagcaaccatttaagaagaccactggagcagctcaagaggaagatgcttgtagctgccgatgtccacaggaagaagaaggaggaggaggaggctatgagctgagagcaaaattcagcaggagtgcagagactgctgccaacctgcaggaccccaaccagctctacaatgagctcaatctagggcgaagagaggaatatgacgtcttggagaagaagcgggctcgggatccagagatgggaggcaaacagcagaggaggaggaacccccaggaaggcgtatacaatgcactgcagaaagacaagatggcagaagcctacagtgagatcggcacaaaaggcgagaggcggagaggcaaggggcacgatggcctttaccagggtctcagcactgccaccaaggacacctatgatgccctgcatatgcagaccctggcccctcgc